European Patent Application EP 4 190 900 A1, published June 7, 2023. Title: Mutant insect olfactory receptor protein. Applicant: SUMITOMO CHEMICAL COMPANY, LIMITED. The sequence listing filed with the application follows.

SEQUENCE LISTING (75 sequences)

SEQ ID NO: 1 - protein, 385 aa, Drosophila melanogaster
MDSFLQVQKSTIALLGFDLFSENREMWKRPYRAMNVFSIAAIFPFILAAVLHNWKNVLLLADAMVALLITILGLFKFSMILYLRRDFKRLIDKFRLLMSNEAEQGEEYAEILNAANKQDQRMCTLFRTCFLLAWALNSVLPLVRMGLSYWLAGHAEPELPFPCLFPWNIHIIRNYVLSFIWSAFASTGVVLPAVSLDTIFCSFTSNLCAFFKIAQYKVVRFKGGSLKESQATLNKVFALYQTSLDMCNDLNQCYQPIICAQFFISSLQLCMLGYLFSITFAQTEGVYYASFIATIIIQAYIYCYCGENLKTESASFEWAIYDSPWHESLGAGGASTSICRSLLISMMRAHRGFRITGYFFEANMEAFSSIVRTAMSYITMLRSFS

SEQ ID NO: 2 - protein, 401 aa, Bombyx mori
MKLLEKLEDPDRPLLGPNVKALKFWGLLLPESRSKKYFYLFMHFAVTVFTATEYIDVWFVKSDLALLLNNLKITMLATVSVLKVTTFLLWQNAWRDLIGYVSRADLEQRATSDSRKLALINGFTGYCRKITYYYWFLMYTTVAIVTVQPIFKFFSSAAYRLDVQSGNGTYLQVVSSWIPWDKNTLPGYLLASIYQTYAAIYGGGWITSFDTNAIVIMVFFRAELELLRIDCAALFDDEKSFGDMAFMRRLKECHRRHTELVKHSRLFDSCLSPIMLLYMFVCSVMLCVTAYQITIETNPMERFLMTEYLVFGVAQLFMYCWHSNDVLYASQDLSRGPYESAWWSRDVKYRKNLYILVAQFNKVIVFSAGPFTKLTVATFIRILKGAYSYYTLLSQSQMNKT

SEQ ID NO: 3 - protein, 417 aa, Anopheles gambiae
MKLNKLNPRWDAYDRRDSFWLQLLCLKYLGLWPPEDTDQATRNRYIAYGWALRIMFLHLYALTQALYFKDVKDINDIANALFVLMTQVTLIYKLEKFNYNIARIQACLRKLNCTLYHPKQREEFSPVLQSMSGVFWLMIFLMFVAIFTIIMWVMSPAFDNERRLPVPAWFPVDYHHSDIVYGVLFLYQTIGIVMSATYNFSTDTMFSGLMLHINGQIVRLGSMVKKLGHDVPPERQLVATDAEWKEMRKRIDHHSKVYGTMYAKVTECVLFHKDILSFGDEVQDIFQGSIFAQVCASVIIICMTLLQATGDDVTMADLLGCGFYLLVMTSQVFIFCYVGNEISYTTDKFTEFVGFSNYFKFDKRTSQAMIFFLQMTLKDVHIKVGSVLKVTLNLHTFLQIMKLSYSYLAVLQSMESE

SEQ ID NO: 4 - protein, 377 aa, Aedes aegypti
MSVEKILACPIISINARVWRFWSFILKHDYMRYISIIPVTAMTVLMFTDLYRAWGNIGEVIINAYFAVLYFNAVLRVLILVHYHEEYESFLEKIADVYREIISMPDEKTKEMVQLFTKRARVMSVSNLGLGAFISACFVVYPLFTGERRLPYGMHIPGVNKFESPLYEILYVMQAVLTFPGCCMYIPFTSFFASTSLFGLIQIKSLQYRLESFKQNGTGKFNKEQRSQLEAIISDHQRVIAYVGELNGLVTYICLVELLSFGMMLCALLFLLVIIEHYAQLIIVVSYIFMIISQIFAFYWHANEVREESMAIGEAAYSGPWIELDQASKKKLLLVILRSQVPLEISVGNVYPMTLEMFQSLLNASYSYFTLLKRVYS

SEQ ID NO: 5 - DNA, 1158 bp, Drosophila melanogaster
atggacagttttctgcaagtacagaagagcaccattgcccttctgggctttgatctctttagtgaaaatcgagaaatgtggaaacgcccctatagagcaatgaatgtgtttagcatagctgccatttttccctttatcctggcagctgtgctccataattggaagaatgtattgctgctggccgatgccatggtggccctactaataaccattctgggcctattcaagtttagcatgatactttacttacgtcgcgatttcaagcgactgattgacaaatttcgtttgctcatgtcgaatgaggcggaacagggcgaggaatacgccgagattctcaacgcagcaaacaagcaggatcaacgaatgtgcactctgtttaggacttgtttcctcctcgcctgggccttgaatagtgttctgcccctcgtgagaatgggtctcagctattggttagcaggtcatgcagagcccgagttgccttttccctgtctttttccctggaatatccacatcattcgcaattatgttttgagcttcatctggagcgctttcgcctcgacaggtgtggttttacctgctgtcagcttggataccatattctgttccttcaccagcaacctgtgcgccttcttcaaaattgcgcagtacaaggtggttagatttaagggcggatcccttaaagaatcacaggccacattgaacaaagtctttgccctgtaccagaccagcttggatatgtgcaacgatctgaatcagtgctaccaaccgattatctgcgcccagttcttcatttcatctctgcaactctgcatgctgggatatctgttctccattacttttgcccagacagagggcgtctactatgcctcattcatagccacaatcattatacaagcctatatctactgctactgcggggagaacctgaagacggagagtgccagcttcgagtgggccatctacgacagtccgtggcacgagagtttgggtgctggtggagcctctacctcgatctgccgatccttgctgatcagcatgatgcgggctcatcggggattccgcattacgggatactttttcgaggcaaacatggaggccttctcatcgattgttcgcacggcgatgtcctacatcacaatgctgagatcattctcctaa

SEQ ID NO: 6 - DNA, 1206 bp, Bombyx mori
atgaagctcctggagaagctagaggaccccgatcgtcctttactaggaccaaacgtcaaagctttgaagttctgggggcttctgttaccggaaagcagatcaaaaaagtatttttacctatttatgcatttcgctgtgactgttttcactgccactgaatatatagacgtatggtttgttaaatcagacctagctttgttattaaacaatctgaagataacaatgttggcgactgtaagcgttttgaaggttaccacttttttgttgtggcaaaatgcctggcgtgacctcattggttacgtatctcgagctgatttagagcaaagggccacttcggactcgagaaagttggctctgataaacggatttaccggctactgccgcaaaataacgtattattactggttcttgatgtatacgaccgtggcaattgttacagtacaaccaatatttaagtttttttcatcagctgcctacagactggacgtccaatctggaaacggtacatacctgcaagtagtaagttcctggataccgtgggataaaaatactttacccggatacctattggcctctatttaccagacatacgcagccatttatggtggaggctggatcacgtccttcgacaccaatgccatagttataatggtattttttagagctgaattggaactattgaggattgattgtgctgctttatttgatgatgaaaaatctttcggtgatatggcttttatgaggagattgaaagagtgtcatagaagacatacagaacttgtcaaacattctcggctgttcgattcttgtttgtcgccgataatgcttctctacatgtttgtctgctcggtaatgctttgtgtgacggcttaccaaattacaatagaaacaaatccgatggaacggttcctcatgaccgagtatttggttttcggcgtggcccagctattcatgtactgttggcacagtaatgatgttctctatgcgagtcaggatctatccagaggtccttacgagagtgcctggtggtcgagagatgtgaagtaccgcaaaaatttatatatattggtggcgcagtttaacaaggttattgtcttttccgcgggccccttcactaagcttacggtcgccacttttatcaggatcctcaaaggagcctatagttactacacactgctcagtcagtcgcaaatgaataaaacatga

SEQ ID NO: 7 - DNA, 1254 bp, Anopheles gambiae
atgaagctgaacaaactgaacccacggtgggatgcgtacgatcgacgggattcgttctggttgcagttgctttgtttgaaatatttaggcctatggccaccggaagatacggatcaggcaacgcggaaccggtacatcgcgtacggttgggctttgcggatcatgtttctacatctgtacgctctaacgcaagccctatacttcaaggatgtgaaggatattaatgacatcgcaaatgcattgttcgtgcttatgactcaagtgacgttgatctacaagctggaaaagtttaactacaacatcgcacggattcaggcttgtctgcgcaagcttaactgcacactgtatcacccgaaacagcgcgaagaattcagccccgttttacaatcgatgagtggagtgttttggctgatgatctttctcatgtttgtggctatcttcaccatcatcatgtgggttatgtcgccagccttcgacaatgaacgtcgtctgcccgtgccggcctggttcccggtggactatcaccattcggacatagtgtacggtgtactgttcctgtatcaaaccattggaatcgtcatgagcgcaacgtacaacttctcgaccgataccatgttttccggcttgatgctacacataaatggacaaattgtgcggcttggtagtatggttaaaaagcttggacatgacgtccctcccgaacgccaattggtcgcaacggatgcggaatggaaagagatgcgaaagcgcatcgaccatcactccaaagtgtacggtacgatgtacgctaaagtaacggagtgtgtgctgtttcacaaggacatcttaagcttcggcgatgaagtgcaggacattttccaaggatctatcttcgcgcaagtatgcgcgtctgtaattatcatttgtatgacactgctgcaagctaccggggacgatgttacgatggccgatctgctgggctgtgggttctatttgctagtaatgacatcgcaagtgtttattttctgttacgtagggaatgaaatctcctatacgacggataaatttacagagtttgttgggttttccaactacttcaagttcgataagcgtaccagccaagcaatgatattttttctgcaaatgactcttaaagatgttcacatcaaggtgggaagtgtcttgaaggttacgctaaatcttcacacatttttgcagattatgaagctatcgtactcctatctggccgtacttcagagcatggaatcagagtaa

SEQ ID NO: 8 - DNA, 1134 bp, Aedes aegypti
atgtccgtcgagaagatcctggcctgtcctatcatttccatcaatgcccgtgtgtggcgcttttggtccttcattctgaagcacgactacatgcgctacatcagcatcatcccggttactgcgatgacggtgctgatgttcaccgatctgtaccgagcgtggggcaatattggcgaagttattatcaacgcctactttgccgtgctctatttcaacgctgtgttgcgagtgctgattttggtccattaccacgaggagtacgaatcgttcttggagaaaatcgcagacgtgtacagggaaatcatctcaatgccggatgaaaaaaccaaggaaatggttcaactttttacgaaacgtgcacgagtgatgtcggtctccaatctgggtttgggtgcctttatcagcgcctgctttgtggtttatccattatttaccggcgaacgtcgacttccttacggaatgcacatccctggcgtgaataaattcgaatcacctttgtatgagatcctgtatgtgatgcaagctgtgctcacctttcccgggtgctgtatgtacattccgtttacgagtttcttcgcttcgacgtcgctgttcggtttgattcagatcaaatcactgcagtatcggttggagagcttcaagcagaatggcactgggaaatttaataaagaacaacgctctcagctggaagccatcatcagtgaccatcagagggtgattgcctatgttggggagctgaatggtttggtgacgtacatttgtctggtggaacttctatcgttcggcatgatgctctgtgcattgctctttctgttggtcattatcgaacactacgcacagctcatcatcgtggtgtcgtacatcttcatgatcatttcgcagattttcgcattctactggcatgccaatgaggtccgggaagagagcatggccattggggaggcagcctacagtggaccatggattgaactggatcaagcgagcaaaaagaaactgttgttggttatcctccgatcacaagtgccactggaaatatccgttggaaatgtctatcctatgacgttggaaatgtttcaatcattattgaatgcatcttactcatatttcactcttttgaaacgtgtttatagctaa

SEQ ID NO: 9 - DNA, 30 bp, Artificial Sequence
  Primer F
caccatggacagttttctgcaagtacagaa

SEQ ID NO: 10 - DNA, 30 bp, Artificial Sequence
  Primer R
ttaggagaatgatctcagcattgtgatgta

SEQ ID NO: 11 - protein, 385 aa, Artificial Sequence
  DmOR47a RX4S
MDSFLQVQKSTIALLGFDLFSENREMWKRPYRAMNVFSIAAIFPFILAAVLHNWKNVLLLADAMVALLITILGLFKFSMILYLRRDFKRLIDKFRLLMSNEAEQGEEYAEILNAANKQDQRMCTLFRTCFLLAWALNSVLPLVRMGLSYWLAGHAEPELPFPCLFPWNIHIIRNYVLSFIWSAFASTGVVLPAVSLDTIFCSFTSNLCAFFKIAQYKVVRFKGGSLKESQATLNKVFALYQTSLDMCNDLNQCYQPIICAQFFISSLQLCMLGYLFSITFAQTEGVYYASFIATIIIQAYIYCYCGENLKTESASFEWAIYDSPWHESLGAGGASTSICRSLLISMMRAHRGFRITGYFFEANMEAFSSIVSTAMSYITMLRSFS

SEQ ID NO: 12 - DNA, 1158 bp, Artificial Sequence
  DmOR47a ERX4S
atggacagttttctgcaagtacagaagagcaccattgcccttctgggctttgatctctttagtgaaaatcgagaaatgtggaaacgcccctatagagcaatgaatgtgtttagcatagctgccatttttccctttatcctggcagctgtgctccataattggaagaatgtattgctgctggccgatgccatggtggccctactaataaccattctgggcctattcaagtttagcatgatactttacttacgtcgcgatttcaagcgactgattgacaaatttcgtttgctcatgtcgaatgaggcggaacagggcgaggaatacgccgagattctcaacgcagcaaacaagcaggatcaacgaatgtgcactctgtttaggacttgtttcctcctcgcctgggccttgaatagtgttctgcccctcgtgagaatgggtctcagctattggttagcaggtcatgcagagcccgagttgccttttccctgtctttttccctggaatatccacatcattcgcaattatgttttgagcttcatctggagcgctttcgcctcgacaggtgtggttttacctgctgtcagcttggataccatattctgttccttcaccagcaacctgtgcgccttcttcaaaattgcgcagtacaaggtggttagatttaagggcggatcccttaaagaatcacaggccacattgaacaaagtctttgccctgtaccagaccagcttggatatgtgcaacgatctgaatcagtgctaccaaccgattatctgcgcccagttcttcatttcatctctgcaactctgcatgctgggatatctgttctccattacttttgcccagacagagggcgtctactatgcctcattcatagccacaatcattatacaagcctatatctactgctactgcggggagaacctgaagacggagagtgccagcttcgagtgggccatctacgacagtccgtggcacgagagtttgggtgctggtggagcctctacctcgatctgccgatccttgctgatcagcatgatgcgggctcatcggggattccgcattacgggatactttttcgaggcaaacatggaggccttctcatcgattgttagcacggcgatgtcctacatcacaatgctgagatcattctcctaa

SEQ ID NO: 13 - DNA, 35 bp, Artificial Sequence
  Primer F
ccttctcatcgattgttagcacggcgatgtcctac

SEQ ID NO: 14 - DNA, 35 bp, Artificial Sequence
  Primer R
gtaggacatcgccgtgctaacaatcgatgagaagg

SEQ ID NO: 15 - protein, 385 aa, Artificial Sequence
  DmOR47a EVX3L-RX4S
MDSFLQVQKSTIALLGFDLFSENREMWKRPYRAMNVFSIAAIFPFILAAVLHNWKNVLLLADAMVALLITILGLFKFSMILYLRRDFKRLIDKFRLLMSNEAEQGEEYAEILNAANKQDQRMCTLFRTCFLLAWALNSVLPLVRMGLSYWLAGHAEPELPFPCLFPWNIHIIRNYVLSFIWSAFASTGVVLPAVSLDTIFCSFTSNLCAFFKIAQYKVVRFKGGSLKESQATLNKVFALYQTSLDMCNDLNQCYQPIICAQFFISSLQLCMLGYLFSITFAQTEGVYYASFIATIIIQAYIYCYCGENLKTESASFEWAIYDSPWHESLGAGGASTSICRSLLISMMRAHRGFRITGYFFEANMEAFSSILSTAMSYITMLRSFS

SEQ ID NO: 16 - DNA, 1158 bp, Artificial Sequence
  DmOR47a EVX3L-RX4S
atggacagttttctgcaagtacagaagagcaccattgcccttctgggctttgatctctttagtgaaaatcgagaaatgtggaaacgcccctatagagcaatgaatgtgtttagcatagctgccatttttccctttatcctggcagctgtgctccataattggaagaatgtattgctgctggccgatgccatggtggccctactaataaccattctgggcctattcaagtttagcatgatactttacttacgtcgcgatttcaagcgactgattgacaaatttcgtttgctcatgtcgaatgaggcggaacagggcgaggaatacgccgagattctcaacgcagcaaacaagcaggatcaacgaatgtgcactctgtttaggacttgtttcctcctcgcctgggccttgaatagtgttctgcccctcgtgagaatgggtctcagctattggttagcaggtcatgcagagcccgagttgccttttccctgtctttttccctggaatatccacatcattcgcaattatgttttgagcttcatctggagcgctttcgcctcgacaggtgtggttttacctgctgtcagcttggataccatattctgttccttcaccagcaacctgtgcgccttcttcaaaattgcgcagtacaaggtggttagatttaagggcggatcccttaaagaatcacaggccacattgaacaaagtctttgccctgtaccagaccagcttggatatgtgcaacgatctgaatcagtgctaccaaccgattatctgcgcccagttcttcatttcatctctgcaactctgcatgctgggatatctgttctccattacttttgcccagacagagggcgtctactatgcctcattcatagccacaatcattatacaagcctatatctactgctactgcggggagaacctgaagacggagagtgccagcttcgagtgggccatctacgacagtccgtggcacgagagtttgggtgctggtggagcctctacctcgatctgccgatccttgctgatcagcatgatgcgggctcatcggggattccgcattacgggatactttttcgaggcaaacatggaggccttctcatcgattcttagcacggcgatgtcctacatcacaatgctgagatcattctcctaa

SEQ ID NO: 17 - DNA, 32 bp, Artificial Sequence
  Primer F
ccttctcatcgattcttagcacggcgatgtcc

SEQ ID NO: 18 - DNA, 32 bp, Artificial Sequence
  Primer R
ggacatcgccgtgctaagaatcgatgagaagg

SEQ ID NO: 19 - protein, 385 aa, Artificial Sequence
  DmOR47a EVX3L-RX4S+alpha
MDSFLQVQKSTIALLGFDLFSENREMWKRPYRAMNVFSIAAIFPFILAAVLHNWKNVLLLADAMVALLITILGLFKFSMILYLRRDFKRLIDKFRLLMSNEAEQGEEYAEILNAANKQDQRMCTLFRTCFLLAWALNSVLPLVRMGLSYWLAGHAEPELPFPCLFPWNIHIIRNYVLSFIWSAFASTGVVLPAVSLDTIFCSFTSNLCAFFKIAQYKVVRFKGGSLKESQATLNKVFALYQTSLDMCNDLNQCYQPIICAQFFISSLQLCMLGYLFSITFAQTEGVYYASFIATIIIQAYIYCYCGENLKTESASFEWAIYDSPWHESLGAGGASTSICRSLLISMMRAHRGFRITGYFYEANLATFQAILSTAYSYFTLLKTFS

SEQ ID NO: 20 - DNA, 1158 bp, Artificial Sequence
  DmOR47a EVX3L-RX4S+alpha
atggacagttttctgcaagtacagaagagcaccattgcccttctgggctttgatctctttagtgaaaatcgagaaatgtggaaacgcccctatagagcaatgaatgtgtttagcatagctgccatttttccctttatcctggcagctgtgctccataattggaagaatgtattgctgctggccgatgccatggtggccctactaataaccattctgggcctattcaagtttagcatgatactttacttacgtcgcgatttcaagcgactgattgacaaatttcgtttgctcatgtcgaatgaggcggaacagggcgaggaatacgccgagattctcaacgcagcaaacaagcaggatcaacgaatgtgcactctgtttaggacttgtttcctcctcgcctgggccttgaatagtgttctgcccctcgtgagaatgggtctcagctattggttagcaggtcatgcagagcccgagttgccttttccctgtctttttccctggaatatccacatcattcgcaattatgttttgagcttcatctggagcgctttcgcctcgacaggtgtggttttacctgctgtcagcttggataccatattctgttccttcaccagcaacctgtgcgccttcttcaaaattgcgcagtacaaggtggttagatttaagggcggatcccttaaagaatcacaggccacattgaacaaagtctttgccctgtaccagaccagcttggatatgtgcaacgatctgaatcagtgctaccaaccgattatctgcgcccagttcttcatttcatctctgcaactctgcatgctgggatatctgttctccattacttttgcccagacagagggcgtctactatgcctcattcatagccacaatcattatacaagcctatatctactgctactgcggggagaacctgaagacggagagtgccagcttcgagtgggccatctacgacagtccgtggcacgagagtttgggtgctggtggagcctctacctcgatctgccgatccttgctgatcagcatgatgcgggctcatcggggattccgcattacgggatacttttacgaggcaaacttggcgacgttccaggcgattcttagcacggcgtactcctacttcacattgctgaaaacattctcctaa

SEQ ID NO: 21 - protein, 480 aa, Artificial Sequence
  Dm(NT-TM4)AaORCO
MTTSMQPSKYTGLVADLMPNIRAMKYSGLFMHNFTGGSAFMKKVYSSVHLVFLLMQFTFILVNMALNAEEVNELSGNTITTLFFTHCITKFIYLAVNQKNFYRTLNIWNQVNTHPLFAESDARYHSIALAKMRKLFFLVMLTTVASATAWTTITFFGDSVKMVVDHETNSSIPVEIPRLPIKSFYPWNASHGMFYMISFAFQIYYVLFSMIHSNLCDVMFCSWLIFACEQLQHLKNIMKPLMEFSATLDTVVPNSGELFKAGSAEQPKEQEPLPPVTPPQGENMLDMDLRGIYSNRTDFTTTFRPTAGMTFNGGVGPNGLTKKQEMLVRSAIKYWVERHKHIVRLVTAIGDAYGVALLLHMLTTTITLTLLAYQATKIHAVDTYAASVVGYLLYSLGQVFMLCIFGNRLIEESSSVMEAAYSCHWYDGSEEAKTFVQIVCQQCQKAMSISGAKFFTVSLDLFASVLGAMVTYFMVLVQLK

SEQ ID NO: 22 - DNA, 1443 bp, Artificial Sequence
  Dm(NT-TM4)AaORCO
atgacaacctcgatgcagccgagcaagtacacgggcctggtcgccgacctgatgcccaacatccgggcgatgaagtactccggcctgttcatgcacaacttcacgggcggcagtgccttcatgaagaaggtgtactcctccgtgcacctggtgttcctcctcatgcagttcaccttcatcctggtcaacatggccctgaacgccgaggaggtcaacgagctgtcgggcaacacgatcacgaccctcttcttcacccactgcatcacgaagtttatctacctggctgttaaccagaagaatttctacagaacattgaatatatggaaccaggtgaacacgcatcccttgttcgccgagtcggatgctcgttaccattcgatcgcactggcgaagatgaggaagctgttctttctggtgatgctgaccacagtcgcctcggccaccgcctggaccacgatcaccttctttggcgacagcgtaaaaatggtggtggaccatgagacgaactccagcatcccggtggagataccccggctgccgattaagtccttctacccgtggaacgccagccacggcatgttctacatgatcagctttgcctttcagatctactacgtgctcttctcgatgatccactccaatctatgcgacgtgatgttctgctcttggctgatattcgcctgcgagcagctgcagcacttgaagaatatcatgaagcctttgatggaattcagcgccacgctggacaccgtcgtgccaaacagtggggaactgttcaaggctggcagtgcagagcagccgaaggaacaggagccattgccaccagtcacgccgccccagggtgaaaacatgttggacatggatcttcgagggatatatagcaacaggaccgacttcacgaccaccttccggccaactgctggaatgacgttcaacggcggggtcgggccaaatgggttgaccaagaaacaggaaatgctggtacgaagcgccatcaagtactgggtagagagacacaagcatatcgttagactcgtaactgcaattggagacgcctatggtgtagctttgctgctacatatgttgactactactattacgttaactttgctcgcttaccaagcaacaaagatacatgcagtagatacatacgcagcatcagtagtaggttatttgctatattctttaggacaagtctttatgctctgtatatttggaaatcgtctcattgaagagagctcatcagtgatggaagcagcttattcttgtcactggtatgatggatcagaggaggccaaaacatttgtacagattgtttgccagcagtgtcagaaagcgatgtcgatttcaggggcaaagttcttcactgtatctttggatctctttgcttcggtgttgggagctatggttacctacttcatggtgttggtgcaactgaagtga

SEQ ID NO: 23 - DNA, 41 bp, Artificial Sequence
  Primer F
tggaattctgcagatcaccatgaagctcctggagaagctag

SEQ ID NO: 24 - DNA, 41 bp, Artificial Sequence
  Primer R
gccactgtgctggattcatgttttattcatttgcgactgac

SEQ ID NO: 25 - protein, 401 aa, Artificial Sequence
  BmOR56 EIX1Q E
MKLLEKLEDPDRPLLGPNVKALKFWGLLLPESRSKKYFYLFMHFAVTVFTATEYIDVWFVKSDLALLLNNLKITMLATVSVLKVTTFLLWQNAWRDLIGYVSRADLEQRATSDSRKLALINGFTGYCRKITYYYWFLMYTTVAIVTVQPIFKFFSSAAYRLDVQSGNGTYLQVVSSWIPWDKNTLPGYLLASIYQTYAAIYGGGWITSFDTNAIVIMVFFRAELELLRIDCAALFDDEKSFGDMAFMRRLKECHRRHTELVKHSRLFDSCLSPIMLLYMFVCSVMLCVTAYQITIETNPMERFLMTEYLVFGVAQLFMYCWHSNDVLYASQDLSRGPYESAWWSRDVKYRKNLYILVAQFNKVIVFSAGPFTKLTVATFQRILKGAYSYYTLLSQSQMNKT

SEQ ID NO: 26 - DNA, 1206 bp, Artificial Sequence
  BmOR56 EIX1Q
atgaagctcctggagaagctagaggaccccgatcgtcctttactaggaccaaacgtcaaagctttgaagttctgggggcttctgttaccggaaagcagatcaaaaaagtatttttacctatttatgcatttcgctgtgactgttttcactgccactgaatatatagacgtatggtttgttaaatcagacctagctttgttattaaacaatctgaagataacaatgttggcgactgtaagcgttttgaaggttaccacttttttgttgtggcaaaatgcctggcgtgacctcattggttacgtatctcgagctgatttagagcaaagggccacttcggactcgagaaagttggctctgataaacggatttaccggctactgccgcaaaataacgtattattactggttcttgatgtatacgaccgtggcaattgttacagtacaaccaatatttaagtttttttcatcagctgcctacagactggacgtccaatctggaaacggtacatacctgcaagtagtaagttcctggataccgtgggataaaaatactttacccggatacctattggcctctatttaccagacatacgcagccatttatggtggaggctggatcacgtccttcgacaccaatgccatagttataatggtattttttagagctgaattggaactattgaggattgattgtgctgctttatttgatgatgaaaaatctttcggtgatatggcttttatgaggagattgaaagagtgtcatagaagacatacagaacttgtcaaacattctcggctgttcgattcttgtttgtcgccgataatgcttctctacatgtttgtctgctcggtaatgctttgtgtgacggcttaccaaattacaatagaaacaaatccgatggaacggttcctcatgaccgagtatttggttttcggcgtggcccagctattcatgtactgttggcacagtaatgatgttctctatgcgagtcaggatctatccagaggtccttacgagagtgcctggtggtcgagagatgtgaagtaccgcaaaaatttatatatattggtggcgcagtttaacaaggttattgtcttttccgcgggccccttcactaagcttacggtcgccacttttcagaggatcctcaaaggagcctatagttactacacactgctcagtcagtcgcaaatgaataaaacatga

SEQ ID NO: 27 - DNA, 33 bp, Artificial Sequence
  Primer F
cggtcgccacttttcagaggatcctcaaaggag

SEQ ID NO: 28 - DNA, 33 bp, Artificial Sequence
  Primer R
ctcctttgaggatcctctgaaaagtggcgaccg

SEQ ID NO: 29 - protein, 401 aa, Artificial Sequence
  BmOR56 ERX2A
MKLLEKLEDPDRPLLGPNVKALKFWGLLLPESRSKKYFYLFMHFAVTVFTATEYIDVWFVKSDLALLLNNLKITMLATVSVLKVTTFLLWQNAWRDLIGYVSRADLEQRATSDSRKLALINGFTGYCRKITYYYWFLMYTTVAIVTVQPIFKFFSSAAYRLDVQSGNGTYLQVVSSWIPWDKNTLPGYLLASIYQTYAAIYGGGWITSFDTNAIVIMVFFRAELELLRIDCAALFDDEKSFGDMAFMRRLKECHRRHTELVKHSRLFDSCLSPIMLLYMFVCSVMLCVTAYQITIETNPMERFLMTEYLVFGVAQLFMYCWHSNDVLYASQDLSRGPYESAWWSRDVKYRKNLYILVAQFNKVIVFSAGPFTKLTVATFIAILKGAYSYYTLLSQSQMNKT

SEQ ID NO: 30 - DNA, 1206 bp, Artificial Sequence
  BmOR56 ERX2A
atgaagctcctggagaagctagaggaccccgatcgtcctttactaggaccaaacgtcaaagctttgaagttctgggggcttctgttaccggaaagcagatcaaaaaagtatttttacctatttatgcatttcgctgtgactgttttcactgccactgaatatatagacgtatggtttgttaaatcagacctagctttgttattaaacaatctgaagataacaatgttggcgactgtaagcgttttgaaggttaccacttttttgttgtggcaaaatgcctggcgtgacctcattggttacgtatctcgagctgatttagagcaaagggccacttcggactcgagaaagttggctctgataaacggatttaccggctactgccgcaaaataacgtattattactggttcttgatgtatacgaccgtggcaattgttacagtacaaccaatatttaagtttttttcatcagctgcctacagactggacgtccaatctggaaacggtacatacctgcaagtagtaagttcctggataccgtgggataaaaatactttacccggatacctattggcctctatttaccagacatacgcagccatttatggtggaggctggatcacgtccttcgacaccaatgccatagttataatggtattttttagagctgaattggaactattgaggattgattgtgctgctttatttgatgatgaaaaatctttcggtgatatggcttttatgaggagattgaaagagtgtcatagaagacatacagaacttgtcaaacattctcggctgttcgattcttgtttgtcgccgataatgcttctctacatgtttgtctgctcggtaatgctttgtgtgacggcttaccaaattacaatagaaacaaatccgatggaacggttcctcatgaccgagtatttggttttcggcgtggcccagctattcatgtactgttggcacagtaatgatgttctctatgcgagtcaggatctatccagaggtccttacgagagtgcctggtggtcgagagatgtgaagtaccgcaaaaatttatatatattggtggcgcagtttaacaaggttattgtcttttccgcgggccccttcactaagcttacggtcgccacttttatcgcaatcctcaaaggagcctatagttactacacactgctcagtcagtcgcaaatgaataaaacatga

SEQ ID NO: 31 - DNA, 33 bp, Artificial Sequence
  Primer F
gtcgccacttttatcgcaatcctcaaaggagcc

SEQ ID NO: 32 - DNA, 33 bp, Artificial Sequence
  Primer R
ggctcctttgaggattgcgataaaagtggcgac

SEQ ID NO: 33 - protein, 401 aa, Artificial Sequence
  BmOR56 EKX4S
MKLLEKLEDPDRPLLGPNVKALKFWGLLLPESRSKKYFYLFMHFAVTVFTATEYIDVWFVKSDLALLLNNLKITMLATVSVLKVTTFLLWQNAWRDLIGYVSRADLEQRATSDSRKLALINGFTGYCRKITYYYWFLMYTTVAIVTVQPIFKFFSSAAYRLDVQSGNGTYLQVVSSWIPWDKNTLPGYLLASIYQTYAAIYGGGWITSFDTNAIVIMVFFRAELELLRIDCAALFDDEKSFGDMAFMRRLKECHRRHTELVKHSRLFDSCLSPIMLLYMFVCSVMLCVTAYQITIETNPMERFLMTEYLVFGVAQLFMYCWHSNDVLYASQDLSRGPYESAWWSRDVKYRKNLYILVAQFNKVIVFSAGPFTKLTVATFIRILSGAYSYYTLLSQSQMNKT

SEQ ID NO: 34 - DNA, 1206 bp, Artificial Sequence
  BmOR56 EKX4S
atgaagctcctggagaagctagaggaccccgatcgtcctttactaggaccaaacgtcaaagctttgaagttctgggggcttctgttaccggaaagcagatcaaaaaagtatttttacctatttatgcatttcgctgtgactgttttcactgccactgaatatatagacgtatggtttgttaaatcagacctagctttgttattaaacaatctgaagataacaatgttggcgactgtaagcgttttgaaggttaccacttttttgttgtggcaaaatgcctggcgtgacctcattggttacgtatctcgagctgatttagagcaaagggccacttcggactcgagaaagttggctctgataaacggatttaccggctactgccgcaaaataacgtattattactggttcttgatgtatacgaccgtggcaattgttacagtacaaccaatatttaagtttttttcatcagctgcctacagactggacgtccaatctggaaacggtacatacctgcaagtagtaagttcctggataccgtgggataaaaatactttacccggatacctattggcctctatttaccagacatacgcagccatttatggtggaggctggatcacgtccttcgacaccaatgccatagttataatggtattttttagagctgaattggaactattgaggattgattgtgctgctttatttgatgatgaaaaatctttcggtgatatggcttttatgaggagattgaaagagtgtcatagaagacatacagaacttgtcaaacattctcggctgttcgattcttgtttgtcgccgataatgcttctctacatgtttgtctgctcggtaatgctttgtgtgacggcttaccaaattacaatagaaacaaatccgatggaacggttcctcatgaccgagtatttggttttcggcgtggcccagctattcatgtactgttggcacagtaatgatgttctctatgcgagtcaggatctatccagaggtccttacgagagtgcctggtggtcgagagatgtgaagtaccgcaaaaatttatatatattggtggcgcagtttaacaaggttattgtcttttccgcgggccccttcactaagcttacggtcgccacttttatcaggatcctcagcggagcctatagttactacacactgctcagtcagtcgcaaatgaataaaacatga

SEQ ID NO: 35 - DNA, 40 bp, Artificial Sequence
  Primer F
cacttttatcaggatcctcagcggagcctatagttactac

SEQ ID NO: 36 - DNA, 40 bp, Artificial Sequence
  Primer R
gtagtaactataggctccgctgaggatcctgataaaagtg

SEQ ID NO: 37 - protein, 401 aa, Artificial Sequence
  BmOR56 EKX4N
MKLLEKLEDPDRPLLGPNVKALKFWGLLLPESRSKKYFYLFMHFAVTVFTATEYIDVWFVKSDLALLLNNLKITMLATVSVLKVTTFLLWQNAWRDLIGYVSRADLEQRATSDSRKLALINGFTGYCRKITYYYWFLMYTTVAIVTVQPIFKFFSSAAYRLDVQSGNGTYLQVVSSWIPWDKNTLPGYLLASIYQTYAAIYGGGWITSFDTNAIVIMVFFRAELELLRIDCAALFDDEKSFGDMAFMRRLKECHRRHTELVKHSRLFDSCLSPIMLLYMFVCSVMLCVTAYQITIETNPMERFLMTEYLVFGVAQLFMYCWHSNDVLYASQDLSRGPYESAWWSRDVKYRKNLYILVAQFNKVIVFSAGPFTKLTVATFIRILNGAYSYYTLLSQSQMNKT

SEQ ID NO: 38 - DNA, 1206 bp, Artificial Sequence
  BmOR56 EKX4N
atgaagctcctggagaagctagaggaccccgatcgtcctttactaggaccaaacgtcaaagctttgaagttctgggggcttctgttaccggaaagcagatcaaaaaagtatttttacctatttatgcatttcgctgtgactgttttcactgccactgaatatatagacgtatggtttgttaaatcagacctagctttgttattaaacaatctgaagataacaatgttggcgactgtaagcgttttgaaggttaccacttttttgttgtggcaaaatgcctggcgtgacctcattggttacgtatctcgagctgatttagagcaaagggccacttcggactcgagaaagttggctctgataaacggatttaccggctactgccgcaaaataacgtattattactggttcttgatgtatacgaccgtggcaattgttacagtacaaccaatatttaagtttttttcatcagctgcctacagactggacgtccaatctggaaacggtacatacctgcaagtagtaagttcctggataccgtgggataaaaatactttacccggatacctattggcctctatttaccagacatacgcagccatttatggtggaggctggatcacgtccttcgacaccaatgccatagttataatggtattttttagagctgaattggaactattgaggattgattgtgctgctttatttgatgatgaaaaatctttcggtgatatggcttttatgaggagattgaaagagtgtcatagaagacatacagaacttgtcaaacattctcggctgttcgattcttgtttgtcgccgataatgcttctctacatgtttgtctgctcggtaatgctttgtgtgacggcttaccaaattacaatagaaacaaatccgatggaacggttcctcatgaccgagtatttggttttcggcgtggcccagctattcatgtactgttggcacagtaatgatgttctctatgcgagtcaggatctatccagaggtccttacgagagtgcctggtggtcgagagatgtgaagtaccgcaaaaatttatatatattggtggcgcagtttaacaaggttattgtcttttccgcgggccccttcactaagcttacggtcgccacttttatcaggatcctcaacggagcctatagttactacacactgctcagtcagtcgcaaatgaataaaacatga

SEQ ID NO: 39 - DNA, 40 bp, Artificial Sequence
  Primer F
cacttttatcaggatcctcaacggagcctatagttactac

SEQ ID NO: 40 - DNA, 40 bp, Artificial Sequence
  Primer R
gtagtaactataggctccgttgaggatcctgataaaagtg

SEQ ID NO: 41 - protein, 401 aa, Artificial Sequence
  BmOR56 EIX1Q-RX2A-KX4S
MKLLEKLEDPDRPLLGPNVKALKFWGLLLPESRSKKYFYLFMHFAVTVFTATEYIDVWFVKSDLALLLNNLKITMLATVSVLKVTTFLLWQNAWRDLIGYVSRADLEQRATSDSRKLALINGFTGYCRKITYYYWFLMYTTVAIVTVQPIFKFFSSAAYRLDVQSGNGTYLQVVSSWIPWDKNTLPGYLLASIYQTYAAIYGGGWITSFDTNAIVIMVFFRAELELLRIDCAALFDDEKSFGDMAFMRRLKECHRRHTELVKHSRLFDSCLSPIMLLYMFVCSVMLCVTAYQITIETNPMERFLMTEYLVFGVAQLFMYCWHSNDVLYASQDLSRGPYESAWWSRDVKYRKNLYILVAQFNKVIVFSAGPFTKLTVATFQAILSGAYSYYTLLSQSQMNKT

SEQ ID NO: 42 - DNA, 1206 bp, Artificial Sequence
  BmOR56 EIX1Q-RX2A-KX4S
atgaagctcctggagaagctagaggaccccgatcgtcctttactaggaccaaacgtcaaagctttgaagttctgggggcttctgttaccggaaagcagatcaaaaaagtatttttacctatttatgcatttcgctgtgactgttttcactgccactgaatatatagacgtatggtttgttaaatcagacctagctttgttattaaacaatctgaagataacaatgttggcgactgtaagcgttttgaaggttaccacttttttgttgtggcaaaatgcctggcgtgacctcattggttacgtatctcgagctgatttagagcaaagggccacttcggactcgagaaagttggctctgataaacggatttaccggctactgccgcaaaataacgtattattactggttcttgatgtatacgaccgtggcaattgttacagtacaaccaatatttaagtttttttcatcagctgcctacagactggacgtccaatctggaaacggtacatacctgcaagtagtaagttcctggataccgtgggataaaaatactttacccggatacctattggcctctatttaccagacatacgcagccatttatggtggaggctggatcacgtccttcgacaccaatgccatagttataatggtattttttagagctgaattggaactattgaggattgattgtgctgctttatttgatgatgaaaaatctttcggtgatatggcttttatgaggagattgaaagagtgtcatagaagacatacagaacttgtcaaacattctcggctgttcgattcttgtttgtcgccgataatgcttctctacatgtttgtctgctcggtaatgctttgtgtgacggcttaccaaattacaatagaaacaaatccgatggaacggttcctcatgaccgagtatttggttttcggcgtggcccagctattcatgtactgttggcacagtaatgatgttctctatgcgagtcaggatctatccagaggtccttacgagagtgcctggtggtcgagagatgtgaagtaccgcaaaaatttatatatattggtggcgcagtttaacaaggttattgtcttttccgcgggccccttcactaagcttacggtcgccacttttcaggcaatcctcagcggagcctatagttactacacactgctcagtcagtcgcaaatgaataaaacatga

SEQ ID NO: 43 - DNA, 40 bp, Artificial Sequence
  Primer F
tggaattctgcagatcaccatgaagctgaacaaactgaac

SEQ ID NO: 44 - DNA, 36 bp, Artificial Sequence
  Primer R
gccactgtgctggatttactctgattccatgctctg

SEQ ID NO: 45 - protein, 417 aa, Artificial Sequence
  AgOR1 EMX3L-KX4S
MKLNKLNPRWDAYDRRDSFWLQLLCLKYLGLWPPEDTDQATRNRYIAYGWALRIMFLHLYALTQALYFKDVKDINDIANALFVLMTQVTLIYKLEKFNYNIARIQACLRKLNCTLYHPKQREEFSPVLQSMSGVFWLMIFLMFVAIFTIIMWVMSPAFDNERRLPVPAWFPVDYHHSDIVYGVLFLYQTIGIVMSATYNFSTDTMFSGLMLHINGQIVRLGSMVKKLGHDVPPERQLVATDAEWKEMRKRIDHHSKVYGTMYAKVTECVLFHKDILSFGDEVQDIFQGSIFAQVCASVIIICMTLLQATGDDVTMADLLGCGFYLLVMTSQVFIFCYVGNEISYTTDKFTEFVGFSNYFKFDKRTSQAMIFFLQMTLKDVHIKVGSVLKVTLNLHTFLQILSLSYSYLAVLQSMESE

SEQ ID NO: 46 - DNA, 1254 bp, Artificial Sequence
  AgOR1 EMX3L-KX4S
atgaagctgaacaaactgaacccacggtgggatgcgtacgatcgacgggattcgttctggttgcagttgctttgtttgaaatatttaggcctatggccaccggaagatacggatcaggcaacgcggaaccggtacatcgcgtacggttgggctttgcggatcatgtttctacatctgtacgctctaacgcaagccctatacttcaaggatgtgaaggatattaatgacatcgcaaatgcattgttcgtgcttatgactcaagtgacgttgatctacaagctggaaaagtttaactacaacatcgcacggattcaggcttgtctgcgcaagcttaactgcacactgtatcacccgaaacagcgcgaagaattcagccccgttttacaatcgatgagtggagtgttttggctgatgatctttctcatgtttgtggctatcttcaccatcatcatgtgggttatgtcgccagccttcgacaatgaacgtcgtctgcccgtgccggcctggttcccggtggactatcaccattcggacatagtgtacggtgtactgttcctgtatcaaaccattggaatcgtcatgagcgcaacgtacaacttctcgaccgataccatgttttccggcttgatgctacacataaatggacaaattgtgcggcttggtagtatggttaaaaagcttggacatgacgtccctcccgaacgccaattggtcgcaacggatgcggaatggaaagagatgcgaaagcgcatcgaccatcactccaaagtgtacggtacgatgtacgctaaagtaacggagtgtgtgctgtttcacaaggacatcttaagcttcggcgatgaagtgcaggacattttccaaggatctatcttcgcgcaagtatgcgcgtctgtaattatcatttgtatgacactgctgcaagctaccggggacgatgttacgatggccgatctgctgggctgtgggttctatttgctagtaatgacatcgcaagtgtttattttctgttacgtagggaatgaaatctcctatacgacggataaatttacagagtttgttgggttttccaactacttcaagttcgataagcgtaccagccaagcaatgatattttttctgcaaatgactcttaaagatgttcacatcaaggtgggaagtgtcttgaaggttacgctaaatcttcacacatttttgcagattttgagcctatcgtactcctatctggccgtacttcagagcatggaatcagagtaa

SEQ ID NO: 47 - DNA, 38 bp, Artificial Sequence
  Primer F
cacatttttgcagattttgagcctatcgtactcctatc

SEQ ID NO: 48 - DNA, 38 bp, Artificial Sequence
  Primer R
gataggagtacgataggctcaaaatctgcaaaaatgtg

SEQ ID NO: 49 - DNA, 38 bp, Artificial Sequence; identical to SEQ ID NO: 47
  Primer F

SEQ ID NO: 50 - DNA, 38 bp, Artificial Sequence; identical to SEQ ID NO: 48
  Primer R

SEQ ID NO: 51 - protein, 417 aa, Artificial Sequence
  AgOR1 EMX3L-KX4N
MKLNKLNPRWDAYDRRDSFWLQLLCLKYLGLWPPEDTDQATRNRYIAYGWALRIMFLHLYALTQALYFKDVKDINDIANALFVLMTQVTLIYKLEKFNYNIARIQACLRKLNCTLYHPKQREEFSPVLQSMSGVFWLMIFLMFVAIFTIIMWVMSPAFDNERRLPVPAWFPVDYHHSDIVYGVLFLYQTIGIVMSATYNFSTDTMFSGLMLHINGQIVRLGSMVKKLGHDVPPERQLVATDAEWKEMRKRIDHHSKVYGTMYAKVTECVLFHKDILSFGDEVQDIFQGSIFAQVCASVIIICMTLLQATGDDVTMADLLGCGFYLLVMTSQVFIFCYVGNEISYTTDKFTEFVGFSNYFKFDKRTSQAMIFFLQMTLKDVHIKVGSVLKVTLNLHTFLQILNLSYSYLAVLQSMESE

SEQ ID NO: 52 - DNA, 1254 bp, Artificial Sequence
  AgOR1 EMX3L-KX4N
atgaagctgaacaaactgaacccacggtgggatgcgtacgatcgacgggattcgttctggttgcagttgctttgtttgaaatatttaggcctatggccaccggaagatacggatcaggcaacgcggaaccggtacatcgcgtacggttgggctttgcggatcatgtttctacatctgtacgctctaacgcaagccctatacttcaaggatgtgaaggatattaatgacatcgcaaatgcattgttcgtgcttatgactcaagtgacgttgatctacaagctggaaaagtttaactacaacatcgcacggattcaggcttgtctgcgcaagcttaactgcacactgtatcacccgaaacagcgcgaagaattcagccccgttttacaatcgatgagtggagtgttttggctgatgatctttctcatgtttgtggctatcttcaccatcatcatgtgggttatgtcgccagccttcgacaatgaacgtcgtctgcccgtgccggcctggttcccggtggactatcaccattcggacatagtgtacggtgtactgttcctgtatcaaaccattggaatcgtcatgagcgcaacgtacaacttctcgaccgataccatgttttccggcttgatgctacacataaatggacaaattgtgcggcttggtagtatggttaaaaagcttggacatgacgtccctcccgaacgccaattggtcgcaacggatgcggaatggaaagagatgcgaaagcgcatcgaccatcactccaaagtgtacggtacgatgtacgctaaagtaacggagtgtgtgctgtttcacaaggacatcttaagcttcggcgatgaagtgcaggacattttccaaggatctatcttcgcgcaagtatgcgcgtctgtaattatcatttgtatgacactgctgcaagctaccggggacgatgttacgatggccgatctgctgggctgtgggttctatttgctagtaatgacatcgcaagtgtttattttctgttacgtagggaatgaaatctcctatacgacggataaatttacagagtttgttgggttttccaactacttcaagttcgataagcgtaccagccaagcaatgatattttttctgcaaatgactcttaaagatgttcacatcaaggtgggaagtgtcttgaaggttacgctaaatcttcacacatttttgcagattttgaacctatcgtactcctatctggccgtacttcagagcatggaatcagagtaa

SEQ ID NO: 53 - DNA, 38 bp, Artificial Sequence
  Primer F
cacatttttgcagattttgaacctatcgtactcctatc

SEQ ID NO: 54 - DNA, 38 bp, Artificial Sequence
  Primer R
gataggagtacgataggttcaaaatctgcaaaaatgtg

SEQ ID NO: 55 - protein, 417 aa, Artificial Sequence
  AgOR1 EMX3L-KX4S+alpha
MKLNKLNPRWDAYDRRDSFWLQLLCLKYLGLWPPEDTDQATRNRYIAYGWALRIMFLHLYALTQALYFKDVKDINDIANALFVLMTQVTLIYKLEKFNYNIARIQACLRKLNCTLYHPKQREEFSPVLQSMSGVFWLMIFLMFVAIFTIIMWVMSPAFDNERRLPVPAWFPVDYHHSDIVYGVLFLYQTIGIVMSATYNFSTDTMFSGLMLHINGQIVRLGSMVKKLGHDVPPERQLVATDAEWKEMRKRIDHHSKVYGTMYAKVTECVLFHKDILSFGDEVQDIFQGSIFAQVCASVIIICMTLLQATGDDVTMADLLGCGFYLLVMTSQVFIFCYVGNEISYTTDKFTEFVGFSNYFKFDKRTSQAMIFFLQMTLKDVHIKVGSVLKVTLNLATFQAILSTAYSYFTLLQSMESE

SEQ ID NO: 56 - DNA, 1254 bp, Artificial Sequence
  AgOR1 EMX3L-KX4S+alpha
atgaagctgaacaaactgaacccacggtgggatgcgtacgatcgacgggattcgttctggttgcagttgctttgtttgaaatatttaggcctatggccaccggaagatacggatcaggcaacgcggaaccggtacatcgcgtacggttgggctttgcggatcatgtttctacatctgtacgctctaacgcaagccctatacttcaaggatgtgaaggatattaatgacatcgcaaatgcattgttcgtgcttatgactcaagtgacgttgatctacaagctggaaaagtttaactacaacatcgcacggattcaggcttgtctgcgcaagcttaactgcacactgtatcacccgaaacagcgcgaagaattcagccccgttttacaatcgatgagtggagtgttttggctgatgatctttctcatgtttgtggctatcttcaccatcatcatgtgggttatgtcgccagccttcgacaatgaacgtcgtctgcccgtgccggcctggttcccggtggactatcaccattcggacatagtgtacggtgtactgttcctgtatcaaaccattggaatcgtcatgagcgcaacgtacaacttctcgaccgataccatgttttccggcttgatgctacacataaatggacaaattgtgcggcttggtagtatggttaaaaagcttggacatgacgtccctcccgaacgccaattggtcgcaacggatgcggaatggaaagagatgcgaaagcgcatcgaccatcactccaaagtgtacggtacgatgtacgctaaagtaacggagtgtgtgctgtttcacaaggacatcttaagcttcggcgatgaagtgcaggacattttccaaggatctatcttcgcgcaagtatgcgcgtctgtaattatcatttgtatgacactgctgcaagctaccggggacgatgttacgatggccgatctgctgggctgtgggttctatttgctagtaatgacatcgcaagtgtttattttctgttacgtagggaatgaaatctcctatacgacggataaatttacagagtttgttgggttttccaactacttcaagttcgataagcgtaccagccaagcaatgatattttttctgcaaatgactcttaaagatgttcacatcaaggtgggaagtgtcttgaaggttacgctaaatcttgccacatttcaggcgattttgagcacagcgtactcctatttcaccctacttcagagcatggaatcagagtaa

SEQ ID NO: 57 - DNA, 42 bp, Artificial Sequence
  Primer F
tggaattctgcagatcaccatgtccgtcgagaagatcctggc

SEQ ID NO: 58 - DNA, 41 bp, Artificial Sequence
  Primer R
gccactgtgctggatttagctataaacacgtttcaaaagag

SEQ ID NO: 59 - protein, 377 aa, Artificial Sequence
  AaOR9 ERX6T
MSVEKILACPIISINARVWRFWSFILKHDYMRYISIIPVTAMTVLMFTDLYRAWGNIGEVIINAYFAVLYFNAVLRVLILVHYHEEYESFLEKIADVYREIISMPDEKTKEMVQLFTKRARVMSVSNLGLGAFISACFVVYPLFTGERRLPYGMHIPGVNKFESPLYEILYVMQAVLTFPGCCMYIPFTSFFASTSLFGLIQIKSLQYRLESFKQNGTGKFNKEQRSQLEAIISDHQRVIAYVGELNGLVTYICLVELLSFGMMLCALLFLLVIIEHYAQLIIVVSYIFMIISQIFAFYWHANEVREESMAIGEAAYSGPWIELDQASKKKLLLVILRSQVPLEISVGNVYPMTLEMFQSLLNASYSYFTLLKTVYS

SEQ ID NO: 60 - DNA, 1134 bp, Artificial Sequence
  AaOR9 ERX6T
atgtccgtcgagaagatcctggcctgtcctatcatttccatcaatgcccgtgtgtggcgcttttggtccttcattctgaagcacgactacatgcgctacatcagcatcatcccggttactgcgatgacggtgctgatgttcaccgatctgtaccgagcgtggggcaatattggcgaagttattatcaacgcctactttgccgtgctctatttcaacgctgtgttgcgagtgctgattttggtccattaccacgaggagtacgaatcgttcttggagaaaatcgcagacgtgtacagggaaatcatctcaatgccggatgaaaaaaccaaggaaatggttcaactttttacgaaacgtgcacgagtgatgtcggtctccaatctgggtttgggtgcctttatcagcgcctgctttgtggtttatccattatttaccggcgaacgtcgacttccttacggaatgcacatccctggcgtgaataaattcgaatcacctttgtatgagatcctgtatgtgatgcaagctgtgctcacctttcccgggtgctgtatgtacattccgtttacgagtttcttcgcttcgacgtcgctgttcggtttgattcagatcaaatcactgcagtatcggttggagagcttcaagcagaatggcactgggaaatttaataaagaacaacgctctcagctggaagccatcatcagtgaccatcagagggtgattgcctatgttggggagctgaatggtttggtgacgtacatttgtctggtggaacttctatcgttcggcatgatgctctgtgcattgctctttctgttggtcattatcgaacactacgcacagctcatcatcgtggtgtcgtacatcttcatgatcatttcgcagattttcgcattctactggcatgccaatgaggtccgggaagagagcatggccattggggaggcagcctacagtggaccatggattgaactggatcaagcgagcaaaaagaaactgttgttggttatcctccgatcacaagtgccactggaaatatccgttggaaatgtctatcctatgacgttggaaatgtttcaatcattattgaatgcatcttactcatatttcactcttttgaaaacggtttatagctaa

SEQ ID NO: 61 - DNA, 37 bp, Artificial Sequence
  Primer F
ctcatatttcactcttttgaaaacggtttatagctaa

SEQ ID NO: 62 - DNA, 37 bp, Artificial Sequence
  Primer R
ttagctataaaccgttttcaaaagagtgaaatatgag

SEQ ID NO: 63 - protein, 377 aa, Artificial Sequence
  AaOR9 ERX6T+alpha
MSVEKILACPIISINARVWRFWSFILKHDYMRYISIIPVTAMTVLMFTDLYRAWGNIGEVIINAYFAVLYFNAVLRVLILVHYHEEYESFLEKIADVYREIISMPDEKTKEMVQLFTKRARVMSVSNLGLGAFISACFVVYPLFTGERRLPYGMHIPGVNKFESPLYEILYVMQAVLTFPGCCMYIPFTSFFASTSLFGLIQIKSLQYRLESFKQNGTGKFNKEQRSQLEAIISDHQRVIAYVGELNGLVTYICLVELLSFGMMLCALLFLLVIIEHYAQLIIVVSYIFMIISQIFAFYWHANEVREESMAIGEAAYSGPWIELDQASKKKLLLVILRSQVPLEISVGKFYPMTLAMFQAILSTAYSYFTLLKTVYS

SEQ ID NO: 64 - DNA, 1134 bp, Artificial Sequence
  AaOR9 ERX6T+alpha
atgtccgtcgagaagatcctggcctgtcctatcatttccatcaatgcccgtgtgtggcgcttttggtccttcattctgaagcacgactacatgcgctacatcagcatcatcccggttactgcgatgacggtgctgatgttcaccgatctgtaccgagcgtggggcaatattggcgaagttattatcaacgcctactttgccgtgctctatttcaacgctgtgttgcgagtgctgattttggtccattaccacgaggagtacgaatcgttcttggagaaaatcgcagacgtgtacagggaaatcatctcaatgccggatgaaaaaaccaaggaaatggttcaactttttacgaaacgtgcacgagtgatgtcggtctccaatctgggtttgggtgcctttatcagcgcctgctttgtggtttatccattatttaccggcgaacgtcgacttccttacggaatgcacatccctggcgtgaataaattcgaatcacctttgtatgagatcctgtatgtgatgcaagctgtgctcacctttcccgggtgctgtatgtacattccgtttacgagtttcttcgcttcgacgtcgctgttcggtttgattcagatcaaatcactgcagtatcggttggagagcttcaagcagaatggcactgggaaatttaataaagaacaacgctctcagctggaagccatcatcagtgaccatcagagggtgattgcctatgttggggagctgaatggtttggtgacgtacatttgtctggtggaacttctatcgttcggcatgatgctctgtgcattgctctttctgttggtcattatcgaacactacgcacagctcatcatcgtggtgtcgtacatcttcatgatcatttcgcagattttcgcattctactggcatgccaatgaggtccgggaagagagcatggccattggggaggcagcctacagtggaccatggattgaactggatcaagcgagcaaaaagaaactgttgttggttatcctccgatcacaagtgccactggaaatatccgttggaaagttctatcctatgacgttggcaatgtttcaagccatcttgagcaccgcctactcatatttcactcttttgaaaacggtttatagctaa

SEQ ID NO: 65 - protein, 398 aa, Anopheles gambiae
MARLVLHEVRYVLMAMLYISRGMAKKIQNSTIDLYVYWFLTFIPIASLCVPQFTYLVVDTKSLIDFISVLVPITEILLTNGKMIICNVKRGKIINLINQVQVAWDECAKSEHLEIQTLITTTAKKSKIFVIIYTTSFLLICVEYSSMPLFKLIYHSAVYGKQSNYTIALPYLSRFAYSTESTTSFAWTYFFILIGVYLLALTLSGFDSLFSTLVMHIKMMFKVLKFEIEQLGLDLSAGKSHVELQAKLKQIILKHKTNLSLIEQLEDGFSFFLMAQFLTSSILVCVVLYELTMVFGWNEDTFKTVTYLPGAILQLFLFCWYAQQITEEARLVSDHIYNIPWYLADPKLQKDILTFMVKAQKPTGVTASKFYMVTLQTFQRISSTSYSYFTLLQTINQQ

SEQ ID NO: 66 - protein, 387 aa, Anopheles gambiae
MVVFDPLDDPLKVLPLPLKLLALLGVNKNPSERFRLYAIYAYLCIALFIPKLCLGYETIPQCFRSIAEGMFSFNTTITFIMLPLKMDNLEDLLKNLKRFTEIVIFNEDYEQILIRLNTAIHKFTKYYFIFTNGVVFAITGSTIAGMLYTYYTKDSEYSAAFPLIMENRLYLIDSHYNLGHCFVHQALMFFALYILLVMFTAKAGTLFGLIRFCSTVLGIIVLKIERLSQIGPVDKYTAELNEIIELHQLAIKCSRQLQNILMEILLAQFTGCVFIWCFMLYYVMISGITAEGIAVVAMLIALSTETFIFCLLGNELTLKGLEISTAMYFTNWYDQPVKLQKMVVPIIQQSQQRIGITAAKFYYIDYNRYGQSLKTAYSFYLLLKDIF

SEQ ID NO: 67 - protein, 423 aa, Anopheles gambiae
MELKEEWILPDVVYANPLLKRTLLGLRYYGILLGQSQSYKKVHCFRGMVFTLSMVLFNCTQYIDLWQVWGSVSDMTANAATTLLFSTTIFRIIFFYFHRARFNSIIKAAHDGIERILKDGWTDEQSIVGSNVRYLKRLAVVFWSCALVTANMMCVYSLVQYLTYEEGPPDGTGTSAANITRKGQPIPPTPILRSWYPTADGKDKHFLEIYLIQLYIMYVGQLIVPSWHMFMVTLMIYGRTECSVLNHRLCFLERYHTAGKDDPTAPVNNAERRSLMIDCIKRQASLVSFTRELEQLTRAAVFLDFVVFSVLLCALLFEASMTPSGVQVFIDVCYITTMTTILFLYYWHANEIHACADRLSMSAYKSDWYRYDRGTNRMLQIFILYSNRPLKMHAFFISMSLDTFLAILRASYSYFTILKQLTD

SEQ ID NO: 68 - protein, 400 aa, Anopheles gambiae
MKPSCKEGVFPLINLSIKLLKIVGFWSKTTGQRISVIGLLAVILYLLAWLIPNWLFIVSSQDNITRLIKATNEQILYFIAFFKLYFYVIHYRRWEKLFYDLQIAFSSVMTNPSPEIQGILGHVTKSTHNLTKYYSYVVNFNCAWYGVFRMLFIVVKYAVTGSYDVPLSTPIEAKYFIPGLHTNFWVWLPVTLGLNVLLEWHSLALVFVETFIWNLVYATSCMFRILQILANELSDRKRNEGIWTVEFEKFSTLHDSVLRSAGTLEEILSGHMLLLYVSTIFSLCLSMVVLSLPIDDFILLLTTFVAFGYCIFQTFSFSYLGTELIEQSEAVADAIFHSKWYTQKLNRQKDMCFLMMRANKPVKLTAAKLFVVTRDSFTQVIKQAYTIFTLMSQFLDNPVN

SEQ ID NO: 69 - protein, 406 aa, Aedes aegypti
MTQSIEFEQTFGFIAKVLQMIGYPSCLAPYPTTFASRLKSSAGFVVCFLMLTYCVFGQIINIGLLMMGYRQTDQVVEEVAIQVSSTGFCIIGLAKMYSLSYNRAILSWLIADFRVKWNAGELTDKDRSIRDGTLRPTVAITTVAALGNIIMVSAFNFQPVVEMIYSRVVTGEWVKLFPYVIWFPFNPTHGAIYYLVYLFEVYSGVIVAVGNVGFNCIFCLLTSHLSMQLKLLCSWIEDMVEVEDEKGVRSKKKLYRIVRYHQDLIRGRNALQSMFSTTLFLNFSASSVLMCMQLYLITTAGITLMVKFTLFMLCILMEIFILCYYGEEILVNSSSIATGAFNSNWYQSKVSQQNPRFGKNLIPIIQRGQRPMVLTAWKFWPITIRTFSAILQTSWSYFTLLRTVMR

SEQ ID NO: 70 - protein, 381 aa, Aedes aegypti
MAPTQNGRDREKFLRVQLLCLALIGIKRHETVSSRTIFHVCFISMVIMDLATILFALEHANDIALVCDCLGPTFTAYLGIVKQYCLSAHRVELWNIIETLRRLKDYAGISEIESIERNNKIDRFLATAYLMSASATGSLFIIAALAKGCYKLIFQNIIEWGFPLSLSFPFKTSHPIVFGMFFVWSSAAIYIVVFCSVSSDASFGGLASNVVVHFKLLQKRLQDATFADNDENLKQLIEYHSLLLNLSRKIMSSFRVIIINNLLVASVLLCVLGFQLVMFLGSTLMLIYLMYVTAIVIQITFFAYYGSLLLHESEEVSISIYCSNWYEASPKTRRILLQCLMRAQVPVNTKAGFMVASLPTLRAILNSAGSYVALLLSFTDN

SEQ ID NO: 71 - protein, 418 aa, Aedes aegypti
MESIRLFVNQVKSKLASLDDESDYFRQMEWAMVVAGIRLPSQNSTYQRLFNCYRILMLLQFSIWVDRVYVAYTEWNSPGELIGVVAFCLALVMILSRVVLMRVYLKDLLKVRDGLENRLNNHHSEGRVRSYRLIRRFFMVLEWIYLFDQIILYAFGINEERQYSVPDNLRRLSKRSKLGFDIFICSNHFVFSSVYASILTIMNTVFMGFSTELENIVSECNGIFERARQQVTVIPLYEGSSEHTEMRENLVFWSTLKNEISLIAERHSELIEHVATVRNLLKVSFLLIFYTEIVFIGCALFYVKLIGITMNTVIVVSYVASILLECYWFCRLTDNINGTNRAIGFALYNLDWPIQLCDLPNSRKQYLEIRASLLVMMTRSQQNLGITCGGMFEMSAQAFDELMKMIYSCLMFLLSVTT

SEQ ID NO: 72 - protein, 419 aa, Aedes aegypti
MATFPIARKRFNYQWLPKMFEIRSLLTHRANNCFWLLDLLLLIAGIRSELTSHWPAECLIRYFANCLFICQYIAGILRLIHALDHEEDGSFLIVCEILIVISLSFACMKVFAINCLRGSLHTLRNFIIGTRVNSGDESFDEFQQLKFFRSARFMMLIVFGLIASDTVLFMIPNRYADVILGLPPQLYMIGKPASSVVNFLLVTFSALGFFPKYLSNVTYIGILLIGMHSKLTSLVHRYRLMLNHPVSSPNQYFEWMSCEVEMVSIQQLEYWNHLRILKNIIGKTFFFVHYFAIFSIGTSGYAIHNVGFNTLSAISLASTLIFLLEYYLLCLWIDKLQDVADSLGSTISELCTKMPYSREYHSKYFGLRASLMITWINTQHAFSMDCMGLFKISTSSFTSLIDTAYTMLMFLTNVCKTEQ

SEQ ID NO: 73 - protein, 378 aa, Anopheles gambiae
MLIEECPIIGVNVRVWLFWSYLRRPRLSRFLVGCIPVAVLNVFQFLKLYSSWGDMSELIINGYFTVLYFNLVLRTSFLVINRRKFETFFEGVAAEYALLEKNDDIRPVLERYTRRGRMLSISNLWLGAFISACFVTYPLFVPGRGLPYGVTIPGVDVLATPTYQVVFVLQVYLTFPACCMYIPFTSFYATCTLFALVQIAALKQRLGRLGRHSGTMASTGHSAGTLFAELKECLKYHKQIIQYVHDLNSLVTHLCLLEFLSFGMMLCALLFLLSISNQLAQMIMIGSYIFMILSQMFAFYWHANEVLEQSLGIGDAIYNGAWPDFEEPIRKRLILIIARAQRPMVIKVGNVYPMTLEMFQKLLNVSYSYFTLLRRVYN

SEQ ID NO: 74 - protein, 375 aa, Anopheles gambiae
MEVLNCPLLSVNVRVWRFWSFVLVHNWRRYISIIPVTALNVFMFADLYRAWGNIEEVIINAYFAVLYFNAVLRTLILVYNRDKYESFLAGAASVYEEIRAINDDVITKLVSTYTKRARFLSISNLALGAFISGCFVVYPLFTGQRGLPYGMFIPGVNNFDSPQYEIFYITQLVLTFPGCCMYIPYTSFFASSTLFGLVQIKTLQHQLKTFRSSEMLNESTVVLNRKLQKLIEDHKRIIRYVQDLNDLVTYICLIEFLSFGLMLCALLFLLNIISVMAQIVIVGAYIFMILTQIFAFYWHSNEVREESMAIAQASYSGPWLNVDDTIKKKLLMMTIRAQRPLEITVGNVYPMTLEMFQSLLNASYSYFTLLRRVYN

SEQ ID NO: 75 - protein, 390 aa, Aedes aegypti
MKYFELTEPEAAMPLALRLLETYGLRGGKRKFLQFQVTILWELLMIVIPKIVFGYRSQDLVIRGLSELLFQLHIMIRISIFAWHRFKYESLIDIIRKVYRKTFSTGGDPTSKSIILKFNQMINKQSKGYFLYIMGCVSLFSVAPVVQSVIIFMANQSRNGTEKAEYVTMMEQEFYGLDIRGNFGHYAIYVALAGLAHYYSASFFAVTGVIIICGVRCTILTFKLINVRLSKLHELPKQDIRDELREIIDLHVDALRCIQLLEQIANLAMVIQIIDCVLIWISMILYMRNNLGVDAISLMVLFVALTGETYALCDLLTQLTSESLAVTRAIIDCQWYSLPLDVQKSLSFVLFRAQRKEGITAAKFFFMDIERFGSVAQTSYSIYVVLKDQL